European Patent Application EP 4 653 011 A1, published November 26, 2025. Title: MRNA VACCINE AND RECOMBINANT PROTEIN VACCINE AGAINST INFECTION BY SARS-COV-2 OR VARIANT THEREOF AND APPLICATIONS THEREOF. Applicant: WestVac Biopharma Co., Ltd. Application CN. The sequence listing filed with the application follows.

SEQUENCE LISTING (8 sequences)

SEQ ID NO: 1 - DNA, 3816 bp, synthetic construct
  source 1..3816: mol_type = other DNA
atgttcgtgttcctggtgctgctgcccctggtgagcagccaatgcgtgaacctgagaacaagaacacagctgccccccgcctacaccaacagcttcacaagaggggtctactaccccgacaaggtgttcagaagcagcgtgctgcacagcacccaagacctgttcctgcccttcttctccaacgtgacctggttccacgccatccacgtgagcggcaccaacggcaccaagagattcgacaaccccgtgctgcccttcaacgacggcgtgtacttcgctagcaccgagaagagcaacatcatcagaggctggatcttcggcaccaccctggacagcaagacacagagcctgctgattgtgaacaacgctaccaacgtggtgatcaaggtgtgcgagtttcagttctgcaacgaccccttcctgggggtgtactaccacaaaaacaacaagagctggatggagagcggcgtgtacagcagcgccaacaactgcaccttcgagtacgtgagccaacccttcctgatggacctggagggcaagcaaggcaacttcaagaacctcagagagttcgtgttcaagaacatcgacggctacttcaagatctacagcaagcacacccccatcaacctggtgagagacctgccccaaggcttcagcgccctggagcccctggtggacctgcccatcggcatcaacatcacaagatttcagaccctgctggccctgcacagaagctacctgacacccggcgacagcagcagcgggtggacagccggcgctgccgcttactacgtgggctacctgcagcctagaaccttcctgctgaagtacaacgagaacggcaccattaccgacgccgtcgactgcgccctggaccccctgagcgagaccaagtgcaccctgaagagcttcaccgtggagaagggcatctatcagacaagcaacttcagagtgcagcccaccgagagcatcgtgagattccccaacatcaccaacctgtgccccttcggcgaggtgttcaacgccacaagattcgctagcgtgtacgcctggaacagaaagagaatcagcaactgcgtggccgactacagcgtgctgtacaacagcgctagcttcagcaccttcaaatgctacggggtcagccccaccaagctgaacgacctgtgcttcaccaacgtgtacgccgacagcttcgtgatcagaggcgacgaggtgagacagatcgcccccgggcagaccggcaagatcgccgactacaactacaagctgcccgacgacttcaccggctgcgtgatcgcctggaactccaacaacctggatagcaaggtgggcggcaactacaactatagatacagactgttcagaaagagcaacctgaagcccttcgagagagacatcagcaccgagatctaccaagccggcagcaagccctgcaacggcgtggagggcttcaactgctacttccccctgcagagctacggctttcagcccaccaacggcgtgggctatcagccctacagagtggtcgtgctgagcttcgagctgctgcacgcccctgccaccgtgtgcggccccaagaagagcaccaacctggtgaagaacaagtgcgtgaacttcaacttcaacggcctgaccggcaccggcgtgctgaccgagagcaacaagaagttcctcccttttcagcagttcggcagagacatcgccgacaccaccgatgccgtgagagaccctcagaccctggagatcctggacatcaccccctgcagctttggcggcgtgagcgtgatcacccccggcaccaacacaagcaaccaagtggccgtgctgtaccaaggcgtgaactgcaccgaggtgcccgtggccatccacgccgatcagctgacccccacctggagagtgtacagcaccggcagcaacgtgtttcagacaagagccggctgcctgatcggcgccgagcacgtgaacaacagctacgagtgcgacatccccatcggcgccggcatctgcgctagctatcagacacagaccaacagcagacggagagctagaagcgtggctagccaaagcatcatcgcctacaccatgagcctgggcgccgagaacagcgtggcctacagcaacaacagcatcgccatccccaccaacttcaccatcagcgtgaccaccgagatcctgcccgtctccatgaccaagacaagcgtggactgcaccatgtacatctgcggcgacagcaccgagtgcagcaacctgctcctgcagtacggcagcttctgcacacagctgaacagagccctgaccggcatcgccgtggagcaagacaagaacacccaagaggtgttcgcccaagtgaagcagatctacaagaccccccccatcaaggacttcggcggcttcaacttcagccaaatcctgcccgaccctagcaagcctagcaagagaagcttcatcgaggacctgctgttcaacaaggtgaccctggccgacgccggcttcatcaagcagtacggcgactgcctgggcgacatcgccgctagagacctgatctgcgctcagaagttcaatggcctgaccgtcctgccccccctgctgaccgacgagatgatcgctcagtacacaagcgccctgctggccggcacaattacaagcggctggacattcggcgctggcgccgccctgcaaatccccttcgccatgcagatggcctacagattcaacggcatcggcgtgacacagaacgtgctgtacgagaatcagaagctgatcgccaatcagttcaacagcgccatcggcaagatccaagacagcctgagcagcaccgctagcgccctgggcaagctgcagaacgtggtgaatcagaacgcccaagccctgaacaccctggtgaagcagctgagcagcaacttcggcgccatcagctccgtgctgaacgatatcctgagcagactggacccccccgaggccgaggtgcagatcgaccggctgatcaccggcagactgcagagcctgcagacctacgtgacacagcagctgatcagagccgccgagatcagagctagcgccaacctggccgccaccaagatgagcgagtgcgtgctggggcagagcaagagagtggacttctgcggcaagggctaccacctgatgagcttccctcagagcgccccccacggcgtggtgttcctgcacgtgacctacgtgcccgcccaagagaagaacttcaccaccgcccccgccatctgccacgacggcaaggcccacttccctagagagggcgtgttcgtgagcaacggcacccactggttcgtgacacagagaaacttctacgagcctcagatcatcaccaccgacaacaccttcgtgagcggcaactgcgacgtggtgatcggcattgtgaacaatacagtctacgaccctctgcagcccgagctggacagcttcaaggaggagctggacaagtacttcaagaatcacacaagccccgacgtggacctgggggacatcagcggcatcaacgctagcgtggtgaacattcagaaggagatcgacagactgaacgaggtggccaagaacctgaacgagagcctgatcgacctgcaagagctgggcaagtacgagcagtacatcaagtggccctggtacatctggctgggcttcatcgccggcctgatcgccatcgtgatggtgaccatcatgctgtgctgcatgacaagctgctgcagctgcctgaagggctgctgctcctgcggcagctgctgcaagttcgacgaggacgacagcgagcccgtgctgaagggcgtgaagctgcactacacctga

SEQ ID NO: 2 - RNA, 3816 nt, synthetic construct
  source 1..3816: mol_type = other RNA
atgttcgtgttcctggtgctgctgcccctggtgagcagccaatgcgtgaacctgagaacaagaacacagctgccccccgcctacaccaacagcttcacaagaggggtctactaccccgacaaggtgttcagaagcagcgtgctgcacagcacccaagacctgttcctgcccttcttctccaacgtgacctggttccacgccatccacgtgagcggcaccaacggcaccaagagattcgacaaccccgtgctgcccttcaacgacggcgtgtacttcgctagcaccgagaagagcaacatcatcagaggctggatcttcggcaccaccctggacagcaagacacagagcctgctgattgtgaacaacgctaccaacgtggtgatcaaggtgtgcgagtttcagttctgcaacgaccccttcctgggggtgtactaccacaaaaacaacaagagctggatggagagcggcgtgtacagcagcgccaacaactgcaccttcgagtacgtgagccaacccttcctgatggacctggagggcaagcaaggcaacttcaagaacctcagagagttcgtgttcaagaacatcgacggctacttcaagatctacagcaagcacacccccatcaacctggtgagagacctgccccaaggcttcagcgccctggagcccctggtggacctgcccatcggcatcaacatcacaagatttcagaccctgctggccctgcacagaagctacctgacacccggcgacagcagcagcgggtggacagccggcgctgccgcttactacgtgggctacctgcagcctagaaccttcctgctgaagtacaacgagaacggcaccattaccgacgccgtcgactgcgccctggaccccctgagcgagaccaagtgcaccctgaagagcttcaccgtggagaagggcatctatcagacaagcaacttcagagtgcagcccaccgagagcatcgtgagattccccaacatcaccaacctgtgccccttcggcgaggtgttcaacgccacaagattcgctagcgtgtacgcctggaacagaaagagaatcagcaactgcgtggccgactacagcgtgctgtacaacagcgctagcttcagcaccttcaaatgctacggggtcagccccaccaagctgaacgacctgtgcttcaccaacgtgtacgccgacagcttcgtgatcagaggcgacgaggtgagacagatcgcccccgggcagaccggcaagatcgccgactacaactacaagctgcccgacgacttcaccggctgcgtgatcgcctggaactccaacaacctggatagcaaggtgggcggcaactacaactatagatacagactgttcagaaagagcaacctgaagcccttcgagagagacatcagcaccgagatctaccaagccggcagcaagccctgcaacggcgtggagggcttcaactgctacttccccctgcagagctacggctttcagcccaccaacggcgtgggctatcagccctacagagtggtcgtgctgagcttcgagctgctgcacgcccctgccaccgtgtgcggccccaagaagagcaccaacctggtgaagaacaagtgcgtgaacttcaacttcaacggcctgaccggcaccggcgtgctgaccgagagcaacaagaagttcctcccttttcagcagttcggcagagacatcgccgacaccaccgatgccgtgagagaccctcagaccctggagatcctggacatcaccccctgcagctttggcggcgtgagcgtgatcacccccggcaccaacacaagcaaccaagtggccgtgctgtaccaaggcgtgaactgcaccgaggtgcccgtggccatccacgccgatcagctgacccccacctggagagtgtacagcaccggcagcaacgtgtttcagacaagagccggctgcctgatcggcgccgagcacgtgaacaacagctacgagtgcgacatccccatcggcgccggcatctgcgctagctatcagacacagaccaacagcagacggagagctagaagcgtggctagccaaagcatcatcgcctacaccatgagcctgggcgccgagaacagcgtggcctacagcaacaacagcatcgccatccccaccaacttcaccatcagcgtgaccaccgagatcctgcccgtctccatgaccaagacaagcgtggactgcaccatgtacatctgcggcgacagcaccgagtgcagcaacctgctcctgcagtacggcagcttctgcacacagctgaacagagccctgaccggcatcgccgtggagcaagacaagaacacccaagaggtgttcgcccaagtgaagcagatctacaagaccccccccatcaaggacttcggcggcttcaacttcagccaaatcctgcccgaccctagcaagcctagcaagagaagcttcatcgaggacctgctgttcaacaaggtgaccctggccgacgccggcttcatcaagcagtacggcgactgcctgggcgacatcgccgctagagacctgatctgcgctcagaagttcaatggcctgaccgtcctgccccccctgctgaccgacgagatgatcgctcagtacacaagcgccctgctggccggcacaattacaagcggctggacattcggcgctggcgccgccctgcaaatccccttcgccatgcagatggcctacagattcaacggcatcggcgtgacacagaacgtgctgtacgagaatcagaagctgatcgccaatcagttcaacagcgccatcggcaagatccaagacagcctgagcagcaccgctagcgccctgggcaagctgcagaacgtggtgaatcagaacgcccaagccctgaacaccctggtgaagcagctgagcagcaacttcggcgccatcagctccgtgctgaacgatatcctgagcagactggacccccccgaggccgaggtgcagatcgaccggctgatcaccggcagactgcagagcctgcagacctacgtgacacagcagctgatcagagccgccgagatcagagctagcgccaacctggccgccaccaagatgagcgagtgcgtgctggggcagagcaagagagtggacttctgcggcaagggctaccacctgatgagcttccctcagagcgccccccacggcgtggtgttcctgcacgtgacctacgtgcccgcccaagagaagaacttcaccaccgcccccgccatctgccacgacggcaaggcccacttccctagagagggcgtgttcgtgagcaacggcacccactggttcgtgacacagagaaacttctacgagcctcagatcatcaccaccgacaacaccttcgtgagcggcaactgcgacgtggtgatcggcattgtgaacaatacagtctacgaccctctgcagcccgagctggacagcttcaaggaggagctggacaagtacttcaagaatcacacaagccccgacgtggacctgggggacatcagcggcatcaacgctagcgtggtgaacattcagaaggagatcgacagactgaacgaggtggccaagaacctgaacgagagcctgatcgacctgcaagagctgggcaagtacgagcagtacatcaagtggccctggtacatctggctgggcttcatcgccggcctgatcgccatcgtgatggtgaccatcatgctgtgctgcatgacaagctgctgcagctgcctgaagggctgctgctcctgcggcagctgctgcaagttcgacgaggacgacagcgagcccgtgctgaagggcgtgaagctgcactacacctga

SEQ ID NO: 3 - protein, 1271 aa, synthetic construct
MFVFLVLLPLVSSQCVNLRTRTQLPPAYTNSFTRGVYYPDKVFRSSVLHSTQDLFLPFFSNVTWFHAIHVSGTNGTKRFDNPVLPFNDGVYFASTEKSNIIRGWIFGTTLDSKTQSLLIVNNATNVVIKVCEFQFCNDPFLGVYYHKNNKSWMESGVYSSANNCTFEYVSQPFLMDLEGKQGNFKNLREFVFKNIDGYFKIYSKHTPINLVRDLPQGFSALEPLVDLPIGINITRFQTLLALHRSYLTPGDSSSGWTAGAAAYYVGYLQPRTFLLKYNENGTITDAVDCALDPLSETKCTLKSFTVEKGIYQTSNFRVQPTESIVRFPNITNLCPFGEVFNATRFASVYAWNRKRISNCVADYSVLYNSASFSTFKCYGVSPTKLNDLCFTNVYADSFVIRGDEVRQIAPGQTGKIADYNYKLPDDFTGCVIAWNSNNLDSKVGGNYNYRYRLFRKSNLKPFERDISTEIYQAGSKPCNGVEGFNCYFPLQSYGFQPTNGVGYQPYRVVVLSFELLHAPATVCGPKKSTNLVKNKCVNFNFNGLTGTGVLTESNKKFLPFQQFGRDIADTTDAVRDPQTLEILDITPCSFGGVSVITPGTNTSNQVAVLYQGVNCTEVPVAIHADQLTPTWRVYSTGSNVFQTRAGCLIGAEHVNNSYECDIPIGAGICASYQTQTNSRRRARSVASQSIIAYTMSLGAENSVAYSNNSIAIPTNFTISVTTEILPVSMTKTSVDCTMYICGDSTECSNLLLQYGSFCTQLNRALTGIAVEQDKNTQEVFAQVKQIYKTPPIKDFGGFNFSQILPDPSKPSKRSFIEDLLFNKVTLADAGFIKQYGDCLGDIAARDLICAQKFNGLTVLPPLLTDEMIAQYTSALLAGTITSGWTFGAGAALQIPFAMQMAYRFNGIGVTQNVLYENQKLIANQFNSAIGKIQDSLSSTASALGKLQNVVNQNAQALNTLVKQLSSNFGAISSVLNDILSRLDPPEAEVQIDRLITGRLQSLQTYVTQQLIRAAEIRASANLAATKMSECVLGQSKRVDFCGKGYHLMSFPQSAPHGVVFLHVTYVPAQEKNFTTAPAICHDGKAHFPREGVFVSNGTHWFVTQRNFYEPQIITTDNTFVSGNCDVVIGIVNNTVYDPLQPELDSFKEELDKYFKNHTSPDVDLGDISGINASVVNIQKEIDRLNEVAKNLNESLIDLQELGKYEQYIKWPWYIWLGFIAGLIAIVMVTIMLCCMTSCCSCLKGCCSCGSCCKFDEDDSEPVLKGVKLHYT

SEQ ID NO: 4 - protein, 492 aa, synthetic construct
MLLVNQSHQGFNKEHTSKMVSAIVLYVLLAAAAHSAFAADSIHIKDSDDLKNRLAEAGDKLVVIDFMATWCGPCKMIGPKLDEMANEMSDSIVVLKVDVDECEDIATEYNINSMPTFVFVKNSKKIEEFSGANVDKLRNTIIKLKLAGSGSGHMHHHHHHSSGDDDDKVQPTESIVRFPNITNLCPFGEVFNATRFASVYAWNRKRISNCVADYSVLYNSASFSTFKCYGVSPTKLNDLCFTNVYADSFVIRGDEVRQIAPGQTGKIADYNYKLPDDFTGCVIAWNSNNLDSKVGGNYNYRYRLFRKSNLKPFERDISTEIYQAGSKPCNGVEGFNCYFPLQSYGFQPTNGVGYQPYRVVVLSFELLHAPATVCGPKKSTNLVKNKSVNFNFNGLYENQKLIANQFNSAIGKIQDSLSSTASALGKLQDVVNQNAQALNTLVKQLKNHTSPDVDLGDISGINASVVNIQKEIDRLNEVAKNLNESLIDLQEL

SEQ ID NO: 5 - DNA, 1479 bp, synthetic construct
  source 1..1479: mol_type = other DNA
atgctactagtaaatcagtcacaccaaggcttcaataaggaacacacaagcaagatggtgagcgctatcgtgctgtacgtcctgctggccgctgctgctcacagcgctttcgctgctgactccatccacatcaaggacagcgacgacctgaagaaccgtctggccgaggccggtgacaagctggtcgtcatcgacttcatggccacttggtgcggtccttgcaagatgatcggccctaagctggacgagatggctaacgagatgtccgacagcatcgtggtcctgaaggtggacgtcgacgagtgcgaggacatcgccaccgaatacaacatcaacagcatgcccaccttcgtgttcgtgaagaacagcaagaagatcgaggaattttccggcgctaacgtcgacaagctgcgtaacaccatcatcaagctgaagctggccggctccggctccggccacatgcatcaccaccaccaccattcctccggtgacgacgacgacaaggtgcagccaaccgaatctatcgtcagattcccaaacatcactaacctgtgccctttcggagaggtgttcaacgctaccaggttcgccagcgtctacgcttggaaccgcaagcgtatcagcaactgcgtcgccgactactctgtgctgtacaactccgctagcttctctactttcaagtgctacggcgtgtcacctaccaagctgaacgacctgtgcttcactaacgtctacgccgactccttcgtgatccgcggagacgaagtccgtcagatcgctcctggacagaccggaaagatcgctgactacaactacaagctgccagacgacttcactggctgcgtgatcgcttggaactcaaacaacctggactccaaggtcggtggcaactacaactaccggtacaggctgttcagaaagtcaaacctgaagcctttcgagcgcgacatctcaaccgaaatctaccaggctggttccaagccctgcaacggtgtggagggcttcaactgctacttccccctgcagtcctacggtttccagccaaccaacggagtcggttaccagccttaccgtgtggtcgtgctgagcttcgaactgctccacgctcctgctactgtgtgcggtcccaagaagtctactaacctggtcaaaaacaaaagcgtcaacttcaacttcaacggtctgtacgagaaccagaagctgatcgctaaccagttcaacagcgccatcggcaagatccaggactcactgtcatccactgcctccgctctgggaaagctgcaggacgtcgtgaaccagaacgcccaggctctgaacaccctggtcaagcagctgaagaaccacacctctcctgacgtcgacctgggcgacatcagcggaatcaacgcttctgtcgtgaacatccagaaggagatcgaccgcctgaacgaagtggccaagaacctgaacgaatccctgattgacctccaagaactctaa

SEQ ID NO: 6 - DNA, 20 bp, synthetic construct
  source 1..20: mol_type = other DNA
gaccccaaaatcagcgaaat

SEQ ID NO: 7 - DNA, 24 bp, synthetic construct
  source 1..24: mol_type = other DNA
tctggttactgccagttgaatctg

SEQ ID NO: 8 - DNA, 24 bp, synthetic construct
  source 1..24: mol_type = other DNA
acnccgcattacgtttggtggacc